European Patent Application EP 4 589 007 A1, published July 23, 2025. Title: PRODUCTION OF VIRAL VECTORS. Applicant: SIRION Biotech GmbH. Application EP. The sequence listing filed with the application follows.

SEQUENCE LISTING (6 sequences)

SEQ ID NO: 1 - DNA, 59 bp, synthetic construct
  source 1..59: mol_type = other DNA
accggcacagtgctaaccagaaaatcatgagattttctggttagcactgtgcttttttg

SEQ ID NO: 2 - DNA, 47 bp, synthetic construct
  source 1..47: mol_type = other DNA
ggaagaatgtgcacagtgctaaccagaaaattcaggacaagactagt

SEQ ID NO: 3 - DNA, 62 bp, synthetic construct
  source 1..62: mol_type = other DNA
accgtacaacagccacaacgtctatatcaagagtatagacgttgtggctgttgtattttttg

SEQ ID NO: 4 - DNA, 43 bp, synthetic construct
  source 1..43: mol_type = other DNA
gaagaatgttacaacagccacaacgtctatattcaggacaaga

SEQ ID NO: 5 - DNA, 132 bp, synthetic construct
  source 1..132: mol_type = other DNA
ctggaggcttgctgaaggctgtatgctgtgtagtatcggatcttggcctgttttggccactgactgacaggccaagccgatactacacaggacacaaggcctgttactagcactcacatggaacaaatggcc

SEQ ID NO: 6 - DNA, 40 bp, synthetic construct
  source 1..40: mol_type = other DNA
taggccaagatccgctactacaattcaggacaagactagt